European Patent Application EP 4 253 534 A2, published October 4, 2023. Title: ALPHA-AMYLASE VARIANTS AND POLYNUCLEOTIDES ENCODING SAME. Applicant: Novozymes A/S. Application EP. The sequence listing filed with the application follows.

SEQUENCE LISTING (14 sequences)

SEQ ID NO: 1 - protein, 483 aa, Bacillus licheniformis [sequence omitted]

SEQ ID NO: 2 - protein, 515 aa, Bacillus stearothermophilus
AAPFNGTMMQYFEWYLPDDGTLWTKVANEANNLSSLGITALWLPPAYKGTSRSDVGYGVYDLYDLGEFNQKGTVRTKYGTKAQYLQAIQAAHAAGMQVYADVVFDHKGGADGTEWVDAVEVNPSDRNQEISGTYQIQAWTKFDFPGRGNTYSSFKWRWYHFDGVDWDESRKLSRIYKFRGIGKAWDWEVDTENGNYDYLMYADLDMDHPEVVTELKNWGKWYVNTTNIDGFRLDAVKHIKFSFFPDWLSYVRSQTGKPLFTVGEYWSYDINKLHNYITKTNGTMSLFDAPLHNKFYTASKSGGAFDMRTLMTNTLMKDQPTLAVTFVDNHDTEPGQALQSWVDPWFKPLAYAFILTRQEGYPCVFYGDYYGIPQYNIPSLKSKIDPLLIARRDYAYGTQHDYLDHSDIIGWTREGVTEKPGSGLAALITDGPGGSKWMYVGKQHAGKVFYDLTGNRSDTVTINSDGWGEFKVNGGSVSVWVPRKTTVSTIARPITTRPWTGEFVRWTEPRLVAWP

SEQ ID NO: 3 - protein, 584 aa, Bacillus sp.
ANTAPINETMMQYFEWDLPNDGTLWTKVKNEAANLSSLGITALWLPPAYKGTSQSDVGYGVYDLYDLGEFNQKGTIRTKYGTKTQYIQAIQAAKAAGMQVYADVVFNHKAGADGTEFVDAVEVDPSNRNQETSGTYQIQAWTKFDFPGRGNTYSSFKWRWYHFDGTDWDESRKLNRIYKFRSTGKAWDWEVDTENGNYDYLMFADLDMDHPEVVTELKNWGTWYVNTTNIDGFRLDAVKHIKYSFFPDWLTYVRNQTGKNLFAVGEFWSYDVNKLHNYITKTNGSMSLFDAPLHNNFYTASKSSGYFDMRYLLNNTLMKDQPSLAVTLVDNHDTQPGQSLQSWVEPWFKPLAYAFILTRQEGYPCVFYGDYYGIPKYNIPGLKSKIDPLLIARRDYAYGTQRDYIDHQDIIGWTREGIDTKPNSGLAALITDGPGGSKWMYVGKKHAGKVFYDLTGNRSDTVTINADGWGEFKVNGGSVSIWVAKTSNVTFTVNNATTTSGQNVYVVANIPELGNWNTANAIKMNPSSYPTWKATIALPQGKAIEFKFIKKDQAGNVIWESTSNRTYTVPFSSTGSYTASWNVP

SEQ ID NO: 4 - protein, 584 aa, Bacillus flavothermus
VPVNGTMMQYFEWYLPDDGTLWTKVANNAQSLANLGITALWLPPAYKGTSSSDVGYGVYDLYDLGEFNQKGTVRTKYGTKTQYIQAIQAAHTAGMQVYADVVFNHKAGADGTELVDAVEVNPSDRNQEISGTYQIQAWTKFDFPGRGNTYSSFKWRWYHFDGTDWDESRKLNRIYKFRGTGKAWDWEVDTENGNYDYLMYADLDMDHPEVVSELKNWGKWYVTTTNIDGFRLDAVKHIKYSFFPDWLSYVRTQTQKPLFAVGEFWSYDISKLHNYITKTNGSMSLFDAPLHNNFYIASKSGGYFDMRTLLNNTLMKDQPTLAVTLVDNHDTEPGQSLQSWVEPWFKPLAYAFILTRQEGYPCVFYGDYYGIPKYNIPALKSKLDPLLIARRDYAYGTQHDYIDSADIIGWTREGVAEKANSGLAALITDGPGGSKWMYVGKQHAGKTFYDLTGNRSDTVTINADGWGEFKVNGGSVSIWVPKISTTSQITFTVNNATTVWGQNVYVVGNISQLGNWDPVHAVQMTPSSYPTWTVTIPLLQGQNIQFKFIKKDSAGNVIWEDISNRTYTVPTAASGAYTASWNVP

SEQ ID NO: 5 - protein, 586 aa, Bacillus sp.
GSVPVNGTMMQYFEWYLPDDGTLWTKVANNAQSLANLGITALWLPPAYKGTSSSDVGYGVYDLYDLGEFNQKGTVRTKYGTKTQYIQAIQAAHTAGMQVYADVVFNHKAGADGTELVDAVEVNPSDRNQEISGTYQIQAWTKFDFPGRGNTYSSFKWRWYHFDGTDWDESRKLNRIYKFRGTGKAWDWEVDTENGNYDYLMYADLDMDHPEVVSELKNWGKWYVITTNIDGFRLDAVKHIKYSFFPDWLSYLRTQTQKPLFAVGEFWSYDINKLHNYITKTNGSMSLFDAPLHNNFYIASKSGGYFDMRTLLNNTLMKEQPTLSVTLVDNHDTEPGQSLQSWVEPWFKPLAYAFILTRQEGYPCVFYGDYYGIPKYNIPALKSKLDPLLIARRDYAYGTQHDYIDNADIIGWTREGVAEKANSGLAALITDGPGGSKWMYVGKQHAGKTFYDLTGNRSDTVTINADGWGEFKVNGGSVSIWVPKTSTTSQITFTVNNATTVWGQNVYVVGNISQLGNWDPVNAVQMTPSSYPTWVVTVPLPQSQNIQFKFIKKDGSGNVIWENISNRTYTVPTAASGAYTANWNVP

SEQ ID NO: 6 - protein, 483 aa, Bacillus amyloliquefaciens
VNGTLMQYFEWYTPNDGQHWKRLQNDAEHLSDIGITAVWIPPAYKGLSQSDNGYGPYDLYDLGEFQQKGTVRTKYGTKSELQDAIGSLHSRNVQVYGDVVLNHKAGADATEDVTAVEVNPANRNQETSEEYQIKAWTDFRFPGRGNTYSDFKWHWYHFDGADWDESRKISRIFKFRGEGKAWDWEVSSENGNYDYLMYADVDYDHPDVVAETKKWGIWYANELSLDGFRIDAAKHIKFSFLRDWVQAVRQATGKEMFTVAEYWQNNAGKLENYLNKTSFNQSVFDVPLHFNLQAASSQGGGYDMRRLLDGTVVSRHPEKAVTFVENHDTQPGQSLESTVQTWFKPLAYAFILTRESGYPQVFYGDMYGTKGTSPKEIPSLKDNIEPILKARKEYAYGPQHDYIDHPDVIGWTREGDSSAAKSGLAALITDGPGGSKRMYAGLKNAGETWYDITGNRSDTVKIGSDGWGEFHVNDGSVSIYVQK

SEQ ID NO: 7 - protein, 485 aa, Bacillus sp.
HHNGTNGTMMQYFEWYLPNDGNHWNRLRDDAANLKSKGITAVWIPPAWKGTSQNDVGYGAYDLYDLGEFNQKGTVRTKYGTRNQLQAAVTSLKNNGIQVYGDVVMNHKGGADGTEIVNAVEVNRSNRNQETSGEYAIEAWTKFDFPGRGNNHSSFKWRWYHFDGTDWDQSRQLQNKIYKFRGTGKAWDWEVDTENGNYDYLMYADVDMDHPEVIHELRNWGVWYTNTLNLDGFRIDAVKHIKYSFTRDWLTHVRNTTGKPMFAVAEFWKNDLGAIENYLNKTSWNHSVFDVPLHYNLYNASNSGGYYDMRNILNGSVVQKHPTHAVTFVDNHDSQPGEALESFVQQWFKPLAYALVLTREQGYPSVFYGDYYGIPTHGVPAMKSKIDPLLQARQTFAYGTQHDYFDHHDIIGWTREGNSSHPNSGLATIMSDGPGGNKWMYVGKNKAGQVWRDITGNRTGTVTINADGWGNFSVNGGSVSVWVKQ

SEQ ID NO: 8 - protein, 485 aa, Bacillus halmapalus
HHNGTNGTMMQYFEWHLPNDGNHWNRLRDDASNLRNRGITAIWIPPAWKGTSQNDVGYGAYDLYDLGEFNQKGTVRTKYGTRSQLESAIHALKNNGVQVYGDVVMNHKGGADATENVLAVEVNPNNRNQEISGDYTIEAWTKFDFPGRGNTYSDFKWRWYHFDGVDWDQSRQFQNRIYKFRGDGKAWDWEVDSENGNYDYLMYADVDMDHPEVVNELRRWGEWYTNTLNLDGFRIDAVKHIKYSFTRDWLTHVRNATGKEMFAVAEFWKNDLGALENYLNKTNWNHSVFDVPLHYNLYNASNSGGNYDMAKLLNGTVVQKHPMHAVTFVDNHDSQPGESLESFVQEWFKPLAYALILTREQGYPSVFYGDYYGIPTHSVPAMKAKIDPILEARQNFAYGTQHDYFDHHNIIGWTREGNTTHPNSGLATIMSDGPGGEKWMYVGQNKAGQVWHDITGNKPGTVTINADGWANFSVNGGSVSIWVKR

SEQ ID NO: 9 - protein, 485 aa, Bacillus sp.
HHNGTNGTMMQYFEWYLPNDGNHWNRLRSDASNLKDKGISAVWIPPAWKGASQNDVGYGAYDLYDLGEFNQKGTIRTKYGTRNQLQAAVNALKSNGIQVYGDVVMNHKGGADATEMVRAVEVNPNNRNQEVSGEYTIEAWTKFDFPGRGNTHSNFKWRWYHFDGVDWDQSRKLNNRIYKFRGDGKGWDWEVDTENGNYDYLMYADIDMDHPEVVNELRNWGVWYTNTLGLDGFRIDAVKHIKYSFTRDWINHVRSATGKNMFAVAEFWKNDLGAIENYLNKTNWNHSVFDVPLHYNLYNASKSGGNYDMRQIFNGTVVQRHPMHAVTFVDNHDSQPEEALESFVEEWFKPLAYALTLTREQGYPSVFYGDYYGIPTHGVPAMKSKIDPILEARQKYAYGRQNDYLDHHNIIGWTREGNTAHPNSGLATIMSDGAGGNKWMFVGRNKAGQVWTDITGNRAGTVTINADGWGNFSVNGGSVSIWVNK

SEQ ID NO: 10 - protein, 485 aa, Bacillus sp.
HHNGTNGTMMQYFEWYLPNDGNHWNRLRSDASNLKDKGITAVWIPPAWKGASQNDVGYGAYDLYDLGEFNQKGTVRTKYGTRNQLQAAVTALKSNGIQVYGDVVMNHKGGADATEWVRAVEVNPSNRNQEVSGDYTIEAWTKFDFPGRGNTHSNFKWRWYHFDGVDWDQSRQLQNRIYKFRGDGKGWDWEVDTENGNYDYLMYADIDMDHPEVVNELRNWGVWYTNTLGLDGFRIDAVKHIKYSFTRDWLTHVRNTTGKNMFAVAEFWKNDIGAIENYLSKTNWNHSVFDVPLHYNLYNASRSGGNYDMRQIFNGTVVQRHPTHAVTFVDNHDSQPEEALESFVEEWFKPLACALTLTRDQGYPSVFYGDYYGIPTHGVPAMKSKIDPILEARQKYAYGKQNDYLDHHNMIGWTREGNTAHPNSGLATIMSDGPGGNKWMYVGRNKAGQVWRDITGNRSGTVTINADGWGNFSVNGGSVSIWVNN

SEQ ID NO: 11 - protein, 485 aa, Bacillus sp.
HHNGTNGTMMQYYEWYLPNDGNHWNRLNSDASNLKSKGITAVWIPPAWKGASQNDVGYGAYDLYDLGEFNQKGTVRTKYGTRSQLQAAVTSLKNNGIQVYGDVVMNHKGGADATEMVRAVEVNPNNRNQEVTGEYTIEAWTRFDFPGRGNTHSSFKWRWYHFDGVDWDQSRRLNNRIYKFRGHGKAWDWEVDTENGNYDYLMYADIDMDHPEVVNELRNWGVWYTNTLGLDGFRIDAVKHIKYSFTRDWINHVRSATGKNMFAVAEFWKNDLGAIENYLQKTNWNHSVFDVPLHYNLYNASKSGGNYDMRNIFNGTVVQRHPSHAVTFVDNHDSQPEEALESFVEEWFKPLAYALTLTREQGYPSVFYGDYYGIPTHGVPAMRSKIDPILEARQKYAYGKQNDYLDHHNIIGWTREGNTAHPNSGLATIMSDGAGGSKWMFVGRNKAGQVWSDITGNRTGTVTINADGWANFSVNGGSVSIWVNK

SEQ ID NO: 12 - protein, 480 aa, Bacillus sp.
DGLNGTMMQYYEWHLENDGQHWNRLHDDAAALSDAGITAIWIPPAYKGNSQADVGYGAYDLYDLGEFNQKGTVRTKYGTKAQLERAIGSLKSNDINVYGDVVMNHKMGADFTEAVQAVQVNPTNRWQDISGAYTIDAWTGFDFSGRNNAYSDFKWRWFHFNGVDWDQRYQENHIFRFANTNWNWRVDEENGNYDYLLGSNIDFSHPEVQDELKDWGSWFTDELDLDGYRLDAIKHIPFWYTSDWVRHQRNEADQDLFVVGEYWKDDVGALEFYLDEMNWEMSLFDVPLNYNFYRASQQGGSYDMRNILRGSLVEAHPMHAVTFVDNHDTQPGESLESWVADWFKPLAYATILTREGGYPNVFYGDYYGIPNDNISAKKDMIDELLDARQNYAYGTQHDYFDHWDVVGWTREGSSSRPNSGLATIMSNGPGGSKWMYVGRQNAGQTWTDLTGNNGASVTINGDGWGEFFTNGGSVSVYVNQ

SEQ ID NO: 13 - protein, 483 aa, Bacillus licheniformis
ANLNGTLMQYFEWYMPNDGQHWKRLQNDSAYLAEHGITAVWIPPAYKGTSQADVGYGAYDLYDLGEFHQKGTVRTKYGTKGELQSAIKSLHSRDINVYGDVVINHKGGADATEDVTAVEVDPADRNRVISGEYLIKAWTHFHFPGRGSTYSDFKWYWYHFDGTDWDESRKLNRIYKFQGKYWDWEVSNENGNYDYLMYADIDYDHPDVVAEIKRWGTWYANELQLDGNRLDAVKHIKFSFLRDWVNHVREKTGKEMFTVAEYWQNDLGALENYLNKTNFNHSVFDVPLHYQFYAASTQGGGYDMRKLLNDTVVSKHPLKSVTFVDNHDTQPGQSLESTVQTWFKPLAYAFILTRESGYPQVFYGDMYGTKGDSQREIPALKHKIEPILKARKQYAYGAQHDYFDHHDIVGWTREGDSSVANSGLAALITDGPGGAKRMYVGRQNAGETWYDITGNRSEPVVINSEGWGEFHVNDGSVSIYVQR

SEQ ID NO: 14 - protein, 481 aa, synthetic construct
  REGION 1..481: note = Variant
VNGTLMQYFEWYTPNDGQHWKRLQNDAEHLSDIGITAVWIPPAYKAISQADVGYGAYDLYDLGEFHQKGTVRTKYGTKGELQSAIKSLHSRDINVYGDVVINHKAGADATEDVTAVEVDPADRNRVISGEHLIKAWTHFHFPGRGSTYSDFKWYWYHFDGTDWDESRKLNRIYKFQGKTWDWEVSNEFGNYDYLMYADFDYDHPDVVAEIKRWGTWYANELQLDGFRLDAVKHIKFSFLRDWVNHVREKTGKEMFTVAEYWSNDLGALENYLNKTNFNHSVFDVPLHYQFHAASTQGGGYDMRKLLNGTVVSKHPLKSVTFVDNHDTQPGQSLESTVQTWFKPLAYAFILTRESGYPQVFYGDMYGTKGDSQREIPALKHKIEPILKARKQYAYGAQHDYFDHHDIVGWTREGDSSVANSGLAALITDGPGGAKRMYVGRQNAGETWHDITGNRSEPVVINSEGWGEFHVNGGSVSIYVQR